European Patent Specification EP 3 845 637 B1, published November 13, 2024. Title: METHODS FOR DIRECT CONVERTION OF HUMAN URINE CELLS INTO NEURAL STEM CELLS USING A SYNTHETIC mRNA. Applicant: StemLab, Inc. The sequence listing filed with the application follows.

SEQUENCE LISTING (32 sequences)

SEQ ID NO: 1 - DNA, 19 bp, Artificial Sequence
  SOX1 forward
acacttgaagcccagatgg

SEQ ID NO: 2 - DNA, 20 bp, Artificial Sequence
  SOX1 reverse
ataggctcacttttggacgg

SEQ ID NO: 3 - DNA, 22 bp, Artificial Sequence
  SOX2 forward
tcaggagttgtcaaggcagaga

SEQ ID NO: 4 - DNA, 22 bp, Artificial Sequence
  SOX2 reverse
ccgccgccgatgattgttatta

SEQ ID NO: 5 - DNA, 19 bp, Artificial Sequence
  PAX6 forward
ggctcaaatgcgacttcag

SEQ ID NO: 6 - DNA, 23 bp, Artificial Sequence
  PAX6 reverse
cccttcgattagaaaaccatacc

SEQ ID NO: 7 - DNA, 22 bp, Artificial Sequence
  PLZF forward
tatacagccacgctgcaagcca

SEQ ID NO: 8 - DNA, 22 bp, Artificial Sequence
  PLZF reverse
tggtctccagcatcttcaggca

SEQ ID NO: 9 - DNA, 22 bp, Artificial Sequence
  EMX1 forward
caggcccaggtagttcaatggg

SEQ ID NO: 10 - DNA, 22 bp, Artificial Sequence
  EMX1 reverse
gctcagccttaagccctgtctc

SEQ ID NO: 11 - DNA, 22 bp, Artificial Sequence
  FOXG1 forward
acccgtcaatgacttcgcagag

SEQ ID NO: 12 - DNA, 22 bp, Artificial Sequence
  FOXG1 reverse
agggttggaagaagacccctga

SEQ ID NO: 13 - DNA, 22 bp, Artificial Sequence
  OTX1 forward
ctcaaacaacccccatacggca

SEQ ID NO: 14 - DNA, 22 bp, Artificial Sequence
  OTX1 reverse
ggtagcgagtcttggcgaagag

SEQ ID NO: 15 - DNA, 24 bp, Artificial Sequence
  OTX2 forward
ttcagggctgtgtgaattgtgtga

SEQ ID NO: 16 - DNA, 24 bp, Artificial Sequence
  OTX2 reverse
cagaggtggagttcaaggttgcat

SEQ ID NO: 17 - DNA, 22 bp, Artificial Sequence
  EN1 forward
gagttccaggcaaaccgctaca

SEQ ID NO: 18 - DNA, 22 bp, Artificial Sequence
  EN1 reverse
gttgtacagtccctgggccatg

SEQ ID NO: 19 - DNA, 22 bp, Artificial Sequence
  GBX2 forward
cggttagcagccacctttccat

SEQ ID NO: 20 - DNA, 22 bp, Artificial Sequence
  GBX2 reverse
gacgtgcttcacatggctcaga

SEQ ID NO: 21 - DNA, 20 bp, Artificial Sequence
  HOXB2 forward
gagacccaggagccaaaagc

SEQ ID NO: 22 - DNA, 20 bp, Artificial Sequence
  HOXB2 reverse
gaaggagacgtggcggattg

SEQ ID NO: 23 - DNA, 22 bp, Artificial Sequence
  HOXB4 forward
ctgagggccagaatgactgctc

SEQ ID NO: 24 - DNA, 22 bp, Artificial Sequence
  HOXB4 reverse
cagaactcaactggcccctcac

SEQ ID NO: 25 - DNA, 20 bp, Artificial Sequence
  VEE forward
acgaagggcaagtcgctgtt

SEQ ID NO: 26 - DNA, 20 bp, Artificial Sequence
  VEE reverse
tttcgtcggcccagttggta

SEQ ID NO: 27 - DNA, 24 bp, Artificial Sequence
  OCT4 forward
gacagggggaggggaggagctagg

SEQ ID NO: 28 - DNA, 26 bp, Artificial Sequence
  OCT4 reverse
cttccctccaaccagttgccccaaac

SEQ ID NO: 29 - DNA, 20 bp, Artificial Sequence
  REX1 forward
ctgaagaaacgggcaaagac

SEQ ID NO: 30 - DNA, 20 bp, Artificial Sequence
  REX1 reverse
gaacattcaagggagcttgc

SEQ ID NO: 31 - DNA, 25 bp, Artificial Sequence
  NANOG forward
cagccctgattcttccaccagtccc

SEQ ID NO: 32 - DNA, 24 bp, Artificial Sequence
  NANOG reverse
ggaaggttcccagtcgggttcacc